European Patent Specification EP 3 828 287 B1, published October 16, 2024. Title: Diagnostic Marker of MCI Due to AD and Uses Thereof. Applicant: SHANGHAI MENTAL HEALTH CENTER (SHANGHAI PSYCHOLOGICAL COUNSELLING TRAINING CENTER). The sequence listing filed with the application follows.

SEQUENCE LISTING (27 sequences)

SEQ ID NO: 1 - DNA, 55 bp, Artificial sequence
  hsa-miR-93-5p
gtcgtatccagtgcgtgtcgtggagtcggcaattgcactggatacgacctacctg

SEQ ID NO: 2 - DNA, 54 bp, Artificial sequence
  hsa-miR-134-3p
gtcgtatccagtgcgtgtcgtggagtcggcaattgcactggatacgacttggtg

SEQ ID NO: 3 - DNA, 55 bp, Artificial sequence
  hsa-miR-34b-5p
gtcgtatccagtgcgtgtcgtggagtcggcaattgcactggatacgaccaatcag

SEQ ID NO: 4 - DNA, 54 bp, Artificial sequence
  hsa-miR-22-5p
gtcgtatccagtgcgtgtcgtggagtcggcaattgcactggatacgactaaagc

SEQ ID NO: 5 - DNA, 56 bp, Artificial sequence
  hsa-miR-1909-3p
gtcgtatccagtgcgtgtcgtggagtcggcaattgcactggatacgaccggtgagc

SEQ ID NO: 6 - DNA, 55 bp, Artificial sequence
  hsa-miR-1185-2-3p
gtcgtatccagtgcgtgtcgtggagtcggcaattgcactggatacgacatgagag

SEQ ID NO: 7 - DNA, 54 bp, Artificial sequence
  hsa-miR-569
gtcgtatccagtgcgtgtcgtggagtcggcaattgcactggatacgacactttc

SEQ ID NO: 8 - DNA, 54 bp, Artificial sequence
  hsa-miR-5691
gtcgtatccagtgcgtgtcgtggagtcggcaattgcactggatacgacgctttc

SEQ ID NO: 9 - DNA, 54 bp, Artificial sequence
  hsa-miR-107
gtcgtatccagtgcgtgtcgtggagtcggcaattgcactggatacgactgatag

SEQ ID NO: 10 - DNA, 18 bp, Artificial sequence
  hsa-miR-93-5p GSP
ggcaaagtgctgttcgtg

SEQ ID NO: 11 - DNA, 18 bp, Artificial sequence
  hsa-miR-93-5p R
cagtgcgtgtcgtggagt

SEQ ID NO: 12 - DNA, 20 bp, Artificial sequence
  hsa-miR-134-3p GSP
gaacctgtgggccacctagt

SEQ ID NO: 13 - DNA, 18 bp, Artificial sequence
  hsa-miR-134-3p R
gtgcgtgtcgtggagtcg

SEQ ID NO: 14 - DNA, 18 bp, Artificial sequence
  hsa-miR-34b-5p GSP
ggggggtaggcagtgtca

SEQ ID NO: 15 - DNA, 18 bp, Artificial sequence
  hsa-miR-34b-5p R
gtgcgtgtcgtggagtcg

SEQ ID NO: 16 - DNA, 20 bp, Artificial sequence
  hsa-miR-22-5p GSP
ggggagttcttcagtggcaa

SEQ ID NO: 17 - DNA, 18 bp, Artificial sequence
  hsa-miR-22-5p R
gtgcgtgtcgtggagtcg

SEQ ID NO: 18 - DNA, 16 bp, Artificial sequence
  hsa-miR-1909-3p GSP
aacgcaggggccgggt

SEQ ID NO: 19 - DNA, 18 bp, Artificial sequence
  hsa-miR-1909-3p R
gtgcgtgtcgtggagtcg

SEQ ID NO: 20 - DNA, 20 bp, Artificial sequence
  hsa-miR-1185-2-3p GSP
ggggaatatacagggggaga

SEQ ID NO: 21 - DNA, 18 bp, Artificial sequence
  hsa-miR-1185-2-3p R
gtgcgtgtcgtggagtcg

SEQ ID NO: 22 - DNA, 22 bp, Artificial sequence
  hsa-miR-569 GSP
ggggggtagttaatgaatcctg

SEQ ID NO: 23 - DNA, 18 bp, Artificial sequence
  hsa-miR-569 R
gtgcgtgtcgtggagtcg

SEQ ID NO: 24 - DNA, 18 bp, Artificial sequence
  hsa-miR-5691 GSP
gcttgctctgagctccga

SEQ ID NO: 25 - DNA, 18 bp, Artificial sequence
  hsa-miR-5691 R
gtgcgtgtcgtggagtcg

SEQ ID NO: 26 - DNA, 18 bp, Artificial sequence
  hsa-miR-107 GSP
ggagcagcattgtacagg

SEQ ID NO: 27 - DNA, 16 bp, Artificial sequence
  hsa-miR-107 R
cagtgcgtgtcgtgga